European Patent Application EP 4 501 958 A1, published February 5, 2025. Title: HRG measuring method using monoclonal antibody against HRG. Applicant: SHIONOGI & CO., LTD. The sequence listing filed with the application follows.

SEQUENCE LISTING (73 sequences)

SEQ ID NO: 1 - protein, 525 aa, Homo sapiens
MKALIAALLLITLQYSCAVSPTDCSAVEPEAEKALDLINKRRRDGYLFQLLRIADAHLDRVENTTVYYLVLDVQESDCSVLSRKYWNDCEPPDSRRPSEIVIGQCKVIATRHSHESQDLRVIDFNCTTSSVSSALANTKDSPVLIDFFEDTERYRKQANKALEKYKEENDDFASFRVDRIERVARVRGGEGTGYFVDFSVRNCPRHHFPRHPNVFGFCRADLFYDVEALDLESPKNLVINCEVFDPQEHENINGVPPHLGHPFHWGGHERSSTTKPPFKPHGSRDHHHPHKPHEHGPPPPPDERDHSHGPPLPQGPPPLLPMSCSSCQHATFGTNGAQRHSHNNNSSDLHPHKHHSHEQHPHGHHPHAHHPHEHDTHRQHPHGHHPHGHHPHGHHPHGHHPHGHHPHCHDFQDYGPCDPPPHNQGHCCHGHGPPPGHLRRRGPGKGPRPFHCRQIGSVYRLPPLRKGEVLPLPEANFPSFPLPHHKHPLKPDNQPFPQSVSESCPGKFKSGFPQVSMFFTHTFPK

SEQ ID NO: 2 - protein, 118 aa, synthetic construct
  REGION 1..118: note = Heavy chain of 3-4E
QVQLQQSGAELMKPGASVKISCKATGYTFSTFWMEWVKQRPGHGLEWIGEILPGSGNANYNEKFKGKATFTADTSSNTAYMQLSSLTSEDSAVYYCAIHYYGYGFAYWGQGTLVTVSA

SEQ ID NO: 3 - protein, 10 aa, synthetic construct
  REGION 1..10: note = CDR1 of 3-4E VH
GYTFSTFWME

SEQ ID NO: 4 - protein, 13 aa, synthetic construct
  REGION 1..13: note = CDR2 of 3-4E VH
EILPGSGNANYNE

SEQ ID NO: 5 - protein, 10 aa, synthetic construct
  REGION 1..10: note = CDR3 of 3-4E VH
IHYYGYGFAY

SEQ ID NO: 6 - protein, 108 aa, synthetic construct
  REGION 1..108: note = Light chain of 3-4E
DNVLTQSPAIMSASLGERVTMTCTASSSVSSSYLHWYQQKPGSSPKLWIYTTSNLASGVPVRFSGSGSGTSYSLTISSMEAEDAATYYCHQYHRSPWTFGGGTKLEIK

SEQ ID NO: 7 - protein, 12 aa, synthetic construct
  REGION 1..12: note = CDR1 of 3-4E VL
TASSSVSSSYLH

SEQ ID NO: 8 - protein, 7 aa, synthetic construct
  REGION 1..7: note = CDR2 of 3-4E VL
TTSNLAS

SEQ ID NO: 9 - protein, 9 aa, synthetic construct
  REGION 1..9: note = CDR3 of 3-4E VL
HQYHRSPWT

SEQ ID NO: 10 - protein, 119 aa, synthetic construct
  REGION 1..119: note = Heavy chain of 6-12A-10B-9G
EVQLQESGPGLVKPSQSLSLTCTVTGYSITSDYAWNWIRQFPGNKLEWMGYISYSGSTNYNPSLRSRISITRDTSKNQFFLQLISVTTEDTATYYCGSASYRYAWFAYWGQGTLVTVSA

SEQ ID NO: 11 - protein, 11 aa, synthetic construct
  REGION 1..11: note = CDR1 of 6-12A-10B-9G VH
GYSITSDYAWN

SEQ ID NO: 12 - protein, 14 aa, synthetic construct
  REGION 1..14: note = CDR2 of 6-12A-10B-9G VH
YISYSGSTNYNPSL

SEQ ID NO: 13 - protein, 10 aa, synthetic construct
  REGION 1..10: note = CDR3 of 6-12A-10B-9G VH
ASYRYAWFAY

SEQ ID NO: 14 - protein, 106 aa, synthetic construct
  REGION 1..106: note = Light chain of 6-12A-10B-9G VL
DIQVTQTTSSLSASLGDRVTISCRASQDISNYLNWYQQKPDGTVKLLIYYTSRLHSGVPSRFSGSGSGTDYSLTISNLEQEDIATYFCQQGNTLPTFGGGTKLEIK

SEQ ID NO: 15 - protein, 11 aa, synthetic construct
  REGION 1..11: note = CDR1 of 6-12A-10B-9G VL
RASQDISNYLN

SEQ ID NO: 16 - protein, 7 aa, synthetic construct
  REGION 1..7: note = CDR2 of 6-12A-10B-9G VL
YTSRLHS

SEQ ID NO: 17 - protein, 8 aa, synthetic construct
  REGION 1..8: note = CDR3 of 6-12A-10B-9G VL
QQGNTLPT

SEQ ID NO: 18 - protein, 119 aa, synthetic construct
  REGION 1..119: note = Heavy chain of 50-6C-2A
EVQLQESGPGLVKPSQSLSLTCTVTGYSITSDYAWNWIRQFPGNKLEWMGYISYSGSTNYNPSLKSRISITRDTSKNQFFLQLNSVTTEDTATYYCASASYRYAWFAYWGQGTLVTVST

SEQ ID NO: 19 - protein, 106 aa, synthetic construct
  REGION 1..106: note = Light chain of 50-6C-2A
DIQMTQTTSSLSASLGDRVTISCRASQDISNYLNWYQQKPDGTVKLLIYYTSRLHSGVPSRFSGSGSGTDYSLTISNLEQEDIGTYFCQQGNTLPTFGGGTKLEIK

SEQ ID NO: 20 - protein, 120 aa, synthetic construct
  REGION 1..120: note = Heavy chain of 65-3A
QVILKESGPGILQPSQTLSLTCSFSGFSLSTSGVGVSWIRQPSGKGLEWLAHIYWDDDKHYNPSLKSRLTISKDTSRNQVFLRITSVDTADTATYYCALGTVGGPWFPYWGQGTLVTVSA

SEQ ID NO: 21 - protein, 12 aa, synthetic construct
  REGION 1..12: note = CDR1 of 65-3A VH
GFSLSTSGVGVS

SEQ ID NO: 22 - protein, 14 aa, synthetic construct
  REGION 1..14: note = CDR2 of 65-3A VH
HIYWDDDKHYNPSL

SEQ ID NO: 23 - protein, 10 aa, synthetic construct
  REGION 1..10: note = CDR3 of 65-3A VH
GTVGGPWFPY

SEQ ID NO: 24 - protein, 107 aa, synthetic construct
  REGION 1..107: note = Light chain of 65-3A
DVQMNQSHKFMSTSVGDRVSITCKASQDVSTAVAWYQQKPGQSPKILIYWASIRHTGVPDRFTGSGSGTDYTLTISSVQAEDLTLYYCQQHYSTPWTFGGGTKLEIK

SEQ ID NO: 25 - protein, 11 aa, synthetic construct
  REGION 1..11: note = CDR1 of 65-3A VL
KASQDVSTAVA

SEQ ID NO: 26 - protein, 7 aa, synthetic construct
  REGION 1..7: note = CDR2 of 65-3A VL
WASIRHT

SEQ ID NO: 27 - protein, 9 aa, synthetic construct
  REGION 1..9: note = CDR3 of 65-3A VL
QQHYSTPWT

SEQ ID NO: 28 - protein, 119 aa, synthetic construct
  REGION 1..119: note = Heavy chain of 67-8A-5F
EVQLQESGPGLVKPSQSLSLTCTVTGYSITSDYAWNWIRQFPGNKLEWMGYISYSGSTSYNPSLKSRISITRDTSKNQFFLQLNSVTTEDTATYYCASASYRYAWFAYWGQGTLVTVSA

SEQ ID NO: 29 - protein, 14 aa, synthetic construct
  REGION 1..14: note = CDR2 of 67-8A-5F VH
YISYSGSTSYNPSL

SEQ ID NO: 30 - protein, 106 aa, synthetic construct
  REGION 1..106: note = Light chain of 67-8A-5F
DIQMTQTTSSLSASLGDRVTISCRASQDISNYLNWYQQKPDGTVKLLIYYTSRLLSGVPSRFSGSGSGTDYSLTISNLEQEDIATYFCQQGNTLPTFGGGTKLEIK

SEQ ID NO: 31 - protein, 7 aa, synthetic construct
  REGION 1..7: note = CDR2 of 67-8A-5F VL
YTSRLLS

SEQ ID NO: 32 - protein, 115 aa, synthetic construct
  REGION 1..115: note = Heavy chain of 69-1A
EVKLEESGGGLVQPGGSMKLSCAASGFTFSDAWMDWVRQSPEKGLEWVAEIRSKANNHGTYYAESVKGRFTISRDDSKSSVYLRMNSLSAEDTGIYYCTRPFAYWGQGTLVTVSA

SEQ ID NO: 33 - protein, 10 aa, synthetic construct
  REGION 1..10: note = CDR1 of 69-1A VH
GFTFSDAWMD

SEQ ID NO: 34 - protein, 17 aa, synthetic construct
  REGION 1..17: note = CDR2 of 69-1A VH
EIRSKANNHGTYYAESV

SEQ ID NO: 35 - protein, 4 aa, synthetic construct
  REGION 1..4: note = CDR3 of 69-1A VH
PFAY

SEQ ID NO: 36 - protein, 112 aa, synthetic construct
  REGION 1..112: note = Light chain of 69-1A
DVVVTQTPLSLPVSLGDQASISCRSSQSLVHIDGNTYFHWYVQKPGQSPKLLIYKVSNRFSGVPDRFSGSGSGTDFTLKISRVEAEDLGVYFCSQSTHVPLTFGAGTKLELK

SEQ ID NO: 37 - protein, 16 aa, synthetic construct
  REGION 1..16: note = CDR1 of 69-1A VL
RSSQSLVHIDGNTYFH

SEQ ID NO: 38 - protein, 7 aa, synthetic construct
  REGION 1..7: note = CDR2 of 69-1A VL
KVSNRFS

SEQ ID NO: 39 - protein, 9 aa, synthetic construct
  REGION 1..9: note = CDR3 of 69-1A VL
SQSTHVPLT

SEQ ID NO: 40 - protein, 118 aa, synthetic construct
  REGION 1..118: note = Heavy chain of 75-2D
QVQLQQSGAELMKPGASVKISCKATGYTFSSYWIEWVKQRPGHGLEWIGEILPGSGRTNYNEKFKGKATFTADTSSNTAYMQLSSLTSEDSAVYYCARYSYFYYFDYWGQGTTLTVSS

SEQ ID NO: 41 - protein, 7 aa, synthetic construct
  REGION 1..7: note = CDR1 of 75-2D VH
GYTFSSY

SEQ ID NO: 42 - protein, 13 aa, synthetic construct
  REGION 1..13: note = CDR2 of 75-2D VH
EILPGSGRTNYNE

SEQ ID NO: 43 - protein, 9 aa, synthetic construct
  REGION 1..9: note = CDR3 of 75-2D VH
YSYFYYFDY

SEQ ID NO: 44 - protein, 108 aa, synthetic construct
  REGION 1..108: note = Light chain of 75-2D
DNVLTQSPAIMSASLGERVTMTCTASSSVSSSYLHWYQQKPGSSPKLWIYSTSNLASGVPARFSGSGSGTSYSLTISSMEAEDAATYYCHQYHRSPWTFGGGTKLEIK

SEQ ID NO: 45 - protein, 7 aa, synthetic construct
  REGION 1..7: note = CDR2 of 75-2D VL
STSNLAS

SEQ ID NO: 46 - protein, 9 aa, synthetic construct
  REGION 1..9: note = CDR3 of 75-2D VL
HQYHRSPWT

SEQ ID NO: 47 - protein, 15 aa, synthetic construct
  REGION 1..15: note = Peptide #1
RDHSHGPPLPQGPPP

SEQ ID NO: 48 - protein, 15 aa, synthetic construct
  REGION 1..15: note = Peptide #2
DHSHGPPLPQGPPPL

SEQ ID NO: 49 - protein, 15 aa, synthetic construct
  REGION 1..15: note = Peptide #3
HSHGPPLPQGPPPLL

SEQ ID NO: 50 - protein, 15 aa, synthetic construct
  REGION 1..15: note = Peptide #4
SHGPPLPQGPPPLLP

SEQ ID NO: 51 - protein, 15 aa, synthetic construct
  REGION 1..15: note = Peptide #5
HGPPLPQGPPPLLPM

SEQ ID NO: 52 - protein, 15 aa, synthetic construct
  REGION 1..15: note = Peptide #6
GPPLPQGPPPLLPMS

SEQ ID NO: 53 - protein, 15 aa, synthetic construct
  REGION 1..15: note = Peptide #7
PPLPQGPPPLLPMSC

SEQ ID NO: 54 - protein, 15 aa, synthetic construct
  REGION 1..15: note = Peptide #8
PLPQGPPPLLPMSCS

SEQ ID NO: 55 - protein, 15 aa, synthetic construct
  REGION 1..15: note = Peptide #9
LPQGPPPLLPMSCSS

SEQ ID NO: 56 - protein, 9 aa, synthetic construct
  REGION 1..9: note = Epitope of 69-1A
PLPQGPPPL

SEQ ID NO: 57 - protein, 15 aa, synthetic construct
  REGION 1..15: note = Peptide #11
HPHGHHPHGHHPHGH

SEQ ID NO: 58 - protein, 15 aa, synthetic construct
  REGION 1..15: note = Peptide #12
PHGHHPHGHHPHGHH

SEQ ID NO: 59 - protein, 15 aa, synthetic construct
  REGION 1..15: note = Peptide #13
HGHHPHGHHPHGHHP

SEQ ID NO: 60 - protein, 15 aa, synthetic construct
  REGION 1..15: note = Peptide #14
GHHPHGHHPHGHHPH

SEQ ID NO: 61 - protein, 15 aa, synthetic construct
  REGION 1..15: note = Peptide #15
HHPHGHHPHGHHPHC

SEQ ID NO: 62 - protein, 15 aa, synthetic construct
  REGION 1..15: note = Peptide #16
HPHGHHPHGHHPHCH

SEQ ID NO: 63 - protein, 15 aa, synthetic construct
  REGION 1..15: note = Peptide #17
PHGHHPHGHHPHCHD

SEQ ID NO: 64 - protein, 15 aa, synthetic construct
  REGION 1..15: note = Peptide #18
HGHHPHGHHPHCHDF

SEQ ID NO: 65 - protein, 15 aa, synthetic construct
  REGION 1..15: note = Peptide #19
GHHPHGHHPHCHDFQ

SEQ ID NO: 66 - protein, 15 aa, synthetic construct
  REGION 1..15: note = Peptide #20
HHPHGHHPHCHDFQD

SEQ ID NO: 67 - protein, 15 aa, synthetic construct
  REGION 1..15: note = Peptide #21
HPHGHHPHCHDFQDY

SEQ ID NO: 68 - protein, 15 aa, synthetic construct
  REGION 1..15: note = Peptide #22
PHGHHPHCHDFQDYG

SEQ ID NO: 69 - protein, 15 aa, synthetic construct
  REGION 1..15: note = Peptide #23
HGHHPHCHDFQDYGP

SEQ ID NO: 70 - protein, 15 aa, synthetic construct
  REGION 1..15: note = Peptide #24
GHHPHCHDFQDYGPC

SEQ ID NO: 71 - protein, 15 aa, synthetic construct
  REGION 1..15: note = Peptide #25
HHPHCHDFQDYGPCD

SEQ ID NO: 72 - protein, 15 aa, synthetic construct
  REGION 1..15: note = Peptide #26
HPHCHDFQDYGPCDP

SEQ ID NO: 73 - protein, 11 aa, synthetic construct
  REGION 1..11: note = Epitope of 75-2D
HPHGHHPHCHD